European Patent Application EP 4 461 306 A1, published November 13, 2024. Title: SNRNA TARGETING USH2A PRE-MRNA AND APPLICATION THEREOF. Applicant: GUANGZHOU REFORGENE MEDICINE CO., LTD. Application CN PCT/CN2022/140599, filed December 21, 2022. The sequence listing filed with the application follows.

SEQUENCE LISTING (46 sequences)

SEQ ID NO: 1 - DNA, 44 bp, synthetic construct
  source 1..44: mol_type = other DNA
cgaagctttaatgatgttggatgtgagccctgccagtgtaacct

SEQ ID NO: 2 - DNA, 32 bp, synthetic construct
  source 1..32: mol_type = other DNA
gagccctgccagtgtaacctccatggctcagt

SEQ ID NO: 3 - DNA, 34 bp, synthetic construct
  source 1..34: mol_type = other DNA
aatcagtggccagtgcctgtgtgtgcctaatcgt

SEQ ID NO: 4 - DNA, 34 bp, synthetic construct
  source 1..34: mol_type = other DNA
taaatatattttatctttagggcttaggtgtgat

SEQ ID NO: 5 - DNA, 29 bp, synthetic construct
  source 1..29: mol_type = other DNA
ctttagggcttaggtgtgatcattgcaat

SEQ ID NO: 6 - DNA, 34 bp, synthetic construct
  source 1..34: mol_type = other DNA
ggtgtgatcattgcaattttggatttaaatttct

SEQ ID NO: 7 - DNA, 34 bp, synthetic construct
  source 1..34: mol_type = other DNA
ttggatttaaatttctccgaagctttaatgatgt

SEQ ID NO: 8 - DNA, 24 bp, synthetic construct
  source 1..24: mol_type = other DNA
agccctaaagataaaatatattta

SEQ ID NO: 9 - DNA, 24 bp, synthetic construct
  source 1..24: mol_type = other DNA
acctaagccctaaagataaaatat

SEQ ID NO: 10 - DNA, 24 bp, synthetic construct
  source 1..24: mol_type = other DNA
atcacacctaagccctaaagataa

SEQ ID NO: 11 - DNA, 24 bp, synthetic construct
  source 1..24: mol_type = other DNA
aatgatcacacctaagccctaaag

SEQ ID NO: 12 - DNA, 24 bp, synthetic construct
  source 1..24: mol_type = other DNA
attgcaatgatcacacctaagccc

SEQ ID NO: 13 - DNA, 24 bp, synthetic construct
  source 1..24: mol_type = other DNA
atccaaaattgcaatgatcacacc

SEQ ID NO: 14 - DNA, 24 bp, synthetic construct
  source 1..24: mol_type = other DNA
atttaaatccaaaattgcaatgat

SEQ ID NO: 15 - DNA, 24 bp, synthetic construct
  source 1..24: mol_type = other DNA
agaaatttaaatccaaaattgcaa

SEQ ID NO: 16 - DNA, 24 bp, synthetic construct
  source 1..24: mol_type = other DNA
agcttcggagaaatttaaatccaa

SEQ ID NO: 17 - DNA, 24 bp, synthetic construct
  source 1..24: mol_type = other DNA
attaaagcttcggagaaatttaaa

SEQ ID NO: 18 - DNA, 24 bp, synthetic construct
  source 1..24: mol_type = other DNA
acatcattaaagcttcggagaaat

SEQ ID NO: 19 - DNA, 24 bp, synthetic construct
  source 1..24: mol_type = other DNA
acatccaacatcattaaagcttcg

SEQ ID NO: 20 - DNA, 24 bp, synthetic construct
  source 1..24: mol_type = other DNA
agggctcacatccaacatcattaa

SEQ ID NO: 21 - DNA, 22 bp, synthetic construct
  source 1..22: mol_type = other DNA
acactggcagggctcacatcca

SEQ ID NO: 22 - DNA, 27 bp, synthetic construct
  source 1..27: mol_type = other DNA
acactggcagggctcacatccaacatc

SEQ ID NO: 23 - DNA, 24 bp, synthetic construct
  source 1..24: mol_type = other DNA
aggttacactggcagggctcacat

SEQ ID NO: 24 - DNA, 24 bp, synthetic construct
  source 1..24: mol_type = other DNA
atggaggttacactggcagggctc

SEQ ID NO: 25 - DNA, 24 bp, synthetic construct
  source 1..24: mol_type = other DNA
actgagccatggaggttacactgg

SEQ ID NO: 26 - DNA, 24 bp, synthetic construct
  source 1..24: mol_type = other DNA
acacacaggcactggccactgatt

SEQ ID NO: 27 - DNA, 24 bp, synthetic construct
  source 1..24: mol_type = other DNA
aggcacacacaggcactggccact

SEQ ID NO: 28 - DNA, 24 bp, synthetic construct
  source 1..24: mol_type = other DNA
acgattaggcacacacaggcactg

SEQ ID NO: 29 - DNA, 20 bp, synthetic construct
  source 1..20: mol_type = other DNA
aggtgtagtcgaccatcgtg

SEQ ID NO: 30 - DNA, 11 bp, synthetic construct
  source 1..11: mol_type = other DNA
aatttgtctag

SEQ ID NO: 31 - DNA, 11 bp, synthetic construct
  source 1..11: mol_type = other DNA
aatttttggag

SEQ ID NO: 32 - DNA, 13 bp, synthetic construct
  source 1..13: mol_type = other DNA
gtctacaatgaaa

SEQ ID NO: 33 - DNA, 66 bp, synthetic construct
  source 1..66: mol_type = other DNA
aggttacactggcagggctcacataatttttggagcaggttttctgacttcggtcggaaaacccct

SEQ ID NO: 34 - DNA, 69 bp, synthetic construct
  source 1..69: mol_type = other DNA
acactggcagggctcacatccaacatcaatttttggagcaggttttctgacttcggtcggaaaacccct

SEQ ID NO: 35 - DNA, 336 bp, synthetic construct
  source 1..336: mol_type = other DNA
atggtgagcaagggcgaggagctgttcaccggggtggtgcccatcctggtcgagctggacggcgacgtaaacggccacaagttcagcgtgtccggcgagggcgagggcgatgccacctacggcaagctgaccctgaagttcatctgcaccaccggcaagctgcccgtgccctggcccaccctcgtgaccaccctgacctacggcgtgcagtgcttcagccgctaccccgaccacatgaagcagcacgacttcttcaagtccgccatgcccgaaggctacgtccaggagcgcaccatcttcttcaaggacgacggcaactacaagacccgcgccgag

SEQ ID NO: 36 - DNA, 384 bp, synthetic construct
  source 1..384: mol_type = other DNA
gtgaagttcgagggcgacaccctggtgaaccgcatcgagctgaagggcatcgacttcaaggaggacggcaacatcctggggcacaagctggagtacaactacaacagccacaacgtctatatcatggccgacaagcagaagaacggcatcaaggtgaacttcaagatccgccacaacatcgaggacggcagcgtgcagctcgccgaccactaccagcagaacacccccatcggcgacggccccgtgctgctgcccgacaaccactacctgagcacccagtccgccctgagcaaagaccccaacgagaagcgcgatcacatggtcctgctggagttcgtgaccgccgccgggatcactctcggcatggacgagctgtacaagtaa

SEQ ID NO: 37 - DNA, 21 bp, synthetic construct
  source 1..21: mol_type = other DNA
agcctttccgccaaggtgatc

SEQ ID NO: 38 - DNA, 21 bp, synthetic construct
  source 1..21: mol_type = other DNA
cacaacgttgcccagcaatgg

SEQ ID NO: 39 - DNA, 26 bp, synthetic construct
  source 1..26: mol_type = other DNA
ccgcaatatgatagggacttagggtg

SEQ ID NO: 40 - DNA, 22 bp, synthetic construct
  source 1..22: mol_type = other DNA
caccctaagtccctatcatatt

SEQ ID NO: 41 - DNA, 22 bp, synthetic construct
  source 1..22: mol_type = other DNA
acactggcagggctcacatcca

SEQ ID NO: 42 - DNA, 48 bp, synthetic construct
  source 1..48: mol_type = other DNA
ccgcaatatgatagggacttagggtgacactggcagggctcacatcca

SEQ ID NO: 43 - DNA, 48 bp, synthetic construct
  source 1..48: mol_type = other DNA
aatttggatgtgagccctgccagtgtcaccctaagtccctatcatatt

SEQ ID NO: 44 - DNA, 91 bp, synthetic construct
  source 1..91: mol_type = other DNA
accgcaatatgatagggacttagggtgacactggcagggctcacatccaaatttttggagcaggttttctgacttcggtcggaaaacccct

SEQ ID NO: 45 - DNA, 20 bp, synthetic construct
  source 1..20: mol_type = other DNA
tatgatagggacttagggtg

SEQ ID NO: 46 - DNA, 437 bp, synthetic construct
  source 1..437: mol_type = other DNA
aagcttaacaacataggagctgtgattggctgttttcagccaatcagcactgactcatttgcatagcctttacaagcggtcacaaactcaagaaacgagcggttttaatagtcttttagaatattgtttatcgaaccgaataaggaactgtgctttgtgattcacatatcagtggaggggtgtggaaatggcaccttgatctcaccctcatcgaaagtggagttgatgtccttccctggctcgctacagacgcacttccgcagagaccaatgtgggtctcgaatttttggagcaggttttctgacttcggtcggaaaacccctcccaatttcactggtctacaatgaaagcaaaacagttctcttccccgctccccggtgtgtgagaggggctttgatccttctctggtttcctaggaaacgcgtatgtgcggccgc